European Patent Application EP 4 166 574 A1, published April 19, 2023. Title: Fusion protein comprising erythropoietin polypeptide. Applicant: BiCA Therapeutics Inc. The sequence listing filed with the application follows.

SEQUENCE LISTING (26 sequences)

SEQ ID NO: 1 - protein, 219 aa, Canis familiaris
APEMLGGPSVFIFPPKPKDTLLIARTPEVTCVVVDLDPEDPEVQISWFVDGKQMQTAKTQPREEQFNGTYRVVSVLPIGHQDWLKGKQFTCKVNNKALPSPIERTISKARGQAHQPSVYVLPPSREELSKNTVSLTCLIKDFFPPDIDVEWQSNGQQEPESKYRTTPPQLDEDGSYFLYSKLSVDKSRWQRGDTFICAVMHEALHNHYTQESLSHSPGK

SEQ ID NO: 2 - protein, 219 aa, Felis catus
PPEMLGGPSIFIFPPKPKDTLSISRTPEVTCLVVDLGPDDSDVQITWFVDNTQVYTAKTSPREEQFNSTYRVVSVLPILHQDWLKGKEFKCKVNSKSLPSPIERTISKAKGQPHEPQVYVLPPAQEELSRNKVSVTCLIKSFHPPDIAVEWEITGQPEPENNYRTTPPQLDSDGTYFVYSKLSVDRSHWQRGNTYTCSVSHEALHSHHTQKSLTQSPGK

SEQ ID NO: 3 - protein, 219 aa, Felis catus
PPEMLGGPSIFIFPPKPKDTLSISRTPEVTCLVVDLGPDDSDVQITWFVDNTQVYTAKTSPREEQFNSTYRVVSVLPILHQDWLKGKEFKCKVNSKSLPSPIERTISKAKGQPHEPQVYVLPPAQEELSRNKVSVTCLIKSFHPPDIAVEWEITGQPEPENNYRTTPPQLDSDGTYFVYSKLSVDRSHWQRGNTYTCSVLHEALHAHHTRKELTQSPGK

SEQ ID NO: 4 - protein, 219 aa, Felis catus
PPEMRRGPKIFIFPPKPKDTLSISRTPEVTCLVVDLGPDDSDVQITWFVDNTQVYTAKTSPREEQFNSTYRVVSVLPILHQDWLKGKEFKCKVNSKSLPSPIERTISKAKGQPHEPQVYVLPPAQEELSRNKVSVTCLIKSFHPPDIAVEWEITGQPEPENNYRTTPPQLDSDGTYFVYSKLSVDRSHWQRGNTYTCSVLHEALHAHHTRKELTQSPGK

SEQ ID NO: 5 - protein, 18 aa, Felis catus
RKTDHPPGPKPGDCPKCP

SEQ ID NO: 6 - protein, 18 aa, Felis catus
RKTDHPPGPKPGDGPKCP

SEQ ID NO: 7 - protein, 18 aa, Felis catus
RKTDHPPGPKPGDCPKGP

SEQ ID NO: 8 - protein, 18 aa, Felis catus
RKTDHPPGPKPGDGPKGP

SEQ ID NO: 9 - protein, 192 aa, Felis catus
MGSCECPALLLLLSLLLLPLGLPVLGAPPRLICDSRVLERYILEAREAENVTMGCAEGPSFSENITVPDTKVNFYTWKRMDVGQQAVEVWQGLALLSEAILRGQALLANSSQPSETLQLHVDKAVSSLRSLTSLLRALGAQKEATSLPEATSAAPLRTFTVDTLCKLFRIYSNFLRGKLTLYTGEACRRGDR

SEQ ID NO: 10 - protein, 192 aa, Felis catus
MGSCECPALLLLLSLLLLPLGLPVLGAPPRLICDSRVLERYILEAREAENVTMGCAEGCSFSENITVPDTKVNFYTWKRMDVGQQAVEVWQGLALLSEAILRGQALLANSSQPSETLQLHVDKAVSSLRSLTSLLRALGAQKEATSLPEATSAAPLRTFTVDTLRKLFRIYSNFLRGKLTLYTGEACRRGDR

SEQ ID NO: 11 - protein, 192 aa, Felis catus
MGSCECPALLLLLSLLLLPLGLPVLGAPPRLICDSRVLERYILEAREAENVTMGCAEGCSFSENITVPDTKVNFYTWKRMDVGQQAVEVWQGLALLSEAILRGQALLANSSQPSETLQLHVDKAVSSLRSLTSLLRALGAQKEATSLPEATSAAPLRTFTVDTLCKLFRIYSNFLRGKLTLYTGEACRRGDR

SEQ ID NO: 12 - protein, 18 aa, Felis catus
RKTDHPPGPKPCDCPKCP

SEQ ID NO: 13 - protein, 429 aa, Felis catus
MGSCECPALLLLLSLLLLPLGLPVLGAPPRLICDSRVLERYILEAREAENVTMGCAEGCSFSENITVPDTKVNFYTWKRMDVGQQAVEVWQGLALLSEAILRGQALLANSSQPSETLQLHVDKAVSSLRSLTSLLRALGAQKEATSLPEATSAAPLRTFTVDTLCKLFRIYSNFLRGKLTLYTGEACRRGDRRKTDHPPGPKPGDCPKCPPPEMLGGPSIFIFPPKPKDTLSISRTPEVTCLVVDLGPDDSDVQITWFVDNTQVYTAKTSPREEQFNSTYRVVSVLPILHQDWLKGKEFKCKVNSKSLPSPIERTISKAKGQPHEPQVYVLPPAQEELSRNKVSVTCLIKSFHPPDIAVEWEITGQPEPENNYRTTPPQLDSDGTYFVYSKLSVDRSHWQRGNTYTCSVSHEALHSHHTQKSLTQSPGK

SEQ ID NO: 14 - protein, 12 aa, Artificial Sequence
  His Tag
GAAHHHHHHHHH

SEQ ID NO: 15 - protein, 192 aa, Mus musculus
MGVPERPTLLLLLSLLLIPLGLPVLCAPPRLICDSRVLERYILEAKEAENVTMGCAEGPRLSENITVPDTKVNFYAWKRMEVEEQAIEVWQGLSLLSEAILQAQALLANSSQPPETLQLHIDKAISGLRSLTSLLRVLGAQKELMSPPDTTPPAPLRTLTVDTFCKLFRVYANFLRGKLKLYTGEVCRRGDR

SEQ ID NO: 16 - protein, 508 aa, Felis catus
MDHLWAPLWPGVGSLCLLLAGAAWAPPPNPLDPKFESKAALLAARGPEELLCFTERLEDLVCFWEEAASAGVGPDNYSFFYQLEGEPWKPCSLHQAPTARGAVRFWCSLPTADASSFVPLELRVTAVSSGAPRYHRIIHINEVVLLDPPAGLLARRADEGGHVVLRWLPPPGAPVASLIRYEVNISSGNVAGGAQKVEILDGRTECALSNLRGRTRYTFMVRARMAEPSFGGFWSAWSEPASLLTASDLDPLILTLSLILVLILLLLAVLALLSHRRTLKQKIWPGIPSPESEFEGLFTTHKGNFQLWLYQNEGCLWWSPCAPFAEDPPSPLEVLSERCWGATQAAEPGAEEGPLLEPLGSEHTQDTYLVLDKWLLPRNPPSEDLPRPDGSLDMVAMHKGSEASSCSSALSLKPGPEGALGASFEYTILDPSSQLLRPRALPPELPPTPPHIKYLYLMVSDSGISTDYSSGGSQEAQGDSSTGPYLNPYENSLIPATETSPPSYVACS

SEQ ID NO: 17 - protein, 507 aa, Mus musculus
MDKLRVPLWPRVGPLCLLLAGAAWAPSPSLPDPKFESKAALLASRGSEELLCFTQRLEDLVCFWEEAASSGMDFNYSFSYQLEGESRKSCSLHQAPTVRGSVRFWCSLPTADTSSFVPLELQVTEASGSPRYHRIIHINEVVLLDAPAGLLARRAEEGSHVVLRWLPPPGAPMTTHIRYEVDVSAGNRAGGTQRVEVLEGRTECVLSNLRGGTRYTFAVRARMAEPSFSGFWSAWSEPASLLTASDLDPLILTLSLILVLISLLLTVLALLSHRRTLQQKIWPGIPSPESEFEGLFTTHKGNFQLWLLQRDGCLWWSPGSSFPEDPPAHLEVLSEPRWAVTQAGDPGADDEGPLLEPVGSEHAQDTYLVLDKWLLPRTPCSENLSGPGGSVDPVTMDEASETSSCPSDLASKPRPEGTSPSSFEYTILDPSSQLLCPRALPPELPPTPPHLKYLYLVVSDSGISTDYSSGGSQGVHGDSSDGPYSHPYENSLVPDSEPLHPGYVACS

SEQ ID NO: 18 - protein, 234 aa, Homo sapiens
EVQLVESGGGLVQPGGSLRLSCAVSGYSITSGYSWNWIRQAPGKGLEWVASITYDGSTNYNPSVKGRITISRDDSKNTFYLQMNSLRAEDTAVYYCARGSHYFGHWHFAVWGQGTLVTVSSASTKGPSVFPLAPSSKSTSGGTAALGCLVKDYFPEPVTVSWNSGALTSGVHTFPAVLQSSGLYSLSSVVTVPSSSLGTQTYICNVNHKPSNTKVDKKVEPKSCDKTHTCPPCP

SEQ ID NO: 19 - protein, 218 aa, Homo sapiens
DIQLTQSPSSLSASVGDRVTITCRASQSVDYDGDSYMNWYQQKPGKAPKLLIYAASYLESGVPSRFSGSGSGTDFTLTISSLQPEDFATYYCQQSHEDPYTFGQGTKVEIKRTVAAPSVFIFPPSDEQLKSGTASVVCLLNNFYPREAKVQWKVDNALQSGNSQESVTEQDSKDSTYSLSSTLTLSKADYEKHKVYACEVTHQGLSSPVTKSFNRGEC

SEQ ID NO: 20 - protein, 19 aa, Artificial Sequence
  secretion signal peptide
MEFGLSWVFLVALFRGVQC

SEQ ID NO: 21 - protein, 22 aa, Artificial Sequence
  secretion signal peptide
MDMRVPAQLLGLLLLWLSGARC

SEQ ID NO: 22 - protein, 297 aa, Canis familiaris
MGVPRPRSWGLGFLLFLLPTLRAADSHLSLLYHLTAVSAPPPGTPAFWASGWLGPQQYLSYNNLRAQAEPYGAWVWENQVSWYWEKETTDLRTKEGLFLEALKALGDGGPYTLQGLLGCELGPDNTSVPVAKFALNGEDFMTFDPKLGTWNGDWPETETVSKRWMQQAGAVSKERTFLLYSCPQRLLGHLERGRGNLEWKEPPSMRLKARPGSPGFSVLTCSAFSFYPPELQLRFLRNGLAAGSGEGDFGPNGDGSFHAWSSLTVKSGDEHHYRCLVQHAGLPQPLTVELESPAKSS

SEQ ID NO: 23 - protein, 297 aa, Felis catus
MGVPRPQPWGLGFLLFLLPTLRAAESHLSLLYHLTAVSSPAPGTPAFWVSGWLGPQQYLSYNNLRAQAEPCGAWVWENQVSWYWEKETTDLRNKQELFLEALKVLGEGGPYTLQGLLGCELGPDNASVPVAKFALNGEDFMDFDPKLGTWSGEWPETETISKRWMQEAGAVSKERTFLLNSCPQRLLGHLERGRGNLEWKEPPSMRLKARPGSPGFSVLTCSAFSFYPPELQLRFLRNGLAAGSGEGDFGPNGDGSFHAWSSLTVKSGDEHHYRCLVQHAGLPQPLTVELESPAKSS

SEQ ID NO: 24 - protein, 8 aa, Artificial Sequence
  His tag
HHHHHHHH

SEQ ID NO: 25 - protein, 125 aa, Canis familiaris
MAPRPALATAGFLALLLILLAACRLDAVQHPPKIQVYSRHPAENGKPNFLNCYVSGFHPPEIEIDLLKNGKEMKAEQTDLSFSKDWTFYLLVHTEFTPNEQDEFSCRVKHVTLSEPQIVKWDRDN

SEQ ID NO: 26 - protein, 118 aa, Felis catus
MARFVVLVLLGLLYLSHLDAVQHSPKVQVYSRHPAENGKPNFLNCYVSGFHPPQIDITLMKNGKKMEAEQTDLSFNRDWTFYLLVHTEFTPTVEDEYSCQVNHTTLSEPKVVKWDRDM